European Patent Application EP 4 494 654 A1, published January 22, 2025. Title: Pharmaceutical Composition of Anti-TIM-3 Antibody and Hypomethylating Agent. Applicant: Nanjing Shunxin Pharmaceuticals Co.,LTD. of Chiatai Tianqing Pharmaceutical Group. Application CN. The sequence listing filed with the application follows.

SEQUENCE LISTING (23 sequences)

SEQ ID NO: 1 - protein, 10 aa, synthetic construct
  source 1..10: note = VH-CDR1 for anti-TIM-3 antibody
GYSFTGYTIN

SEQ ID NO: 2 - protein, 10 aa, synthetic construct
  source 1..10: note = VH-CDR2 for anti-TIM-3 antibody
LFNPYNGGTT

SEQ ID NO: 3 - protein, 10 aa, synthetic construct
  source 1..10: note = VH-CDR3 for anti-TIM-3 antibody
RYYGYDAMDY

SEQ ID NO: 4 - protein, 17 aa, synthetic construct
  source 1..17: note = VL-CDR1 for anti-TIM-3 antibody
KSSQSVLYSSNQKNHLA

SEQ ID NO: 5 - protein, 7 aa, synthetic construct
  source 1..7: note = VL-CDR2 for anti-TIM-3 antibody
WASTRES

SEQ ID NO: 6 - protein, 8 aa, synthetic construct
  source 1..8: note = VL-CDR3 for anti-TIM-3 antibody
HQYLSSYT

SEQ ID NO: 7 - protein, 119 aa, synthetic construct
  source 1..119: note = VH for anti-TIM-3 antibody
QVQLVQSGAEVKKPGASVKVSCKASGYSFTGYTINWVRQAPGQGLEWMGLFNPYNGGTTYAQKFQGRVTMTVDKSTSTVYMELSSLRSEDTAVYYCARRYYGYDAMDYWGQGTLVTVSS

SEQ ID NO: 8 - protein, 112 aa, synthetic construct
  source 1..112: note = VL for anti-TIM-3 antibody
DIQMTQSPSSLSASVGDRVTITCKSSQSVLYSSNQKNHLAWYQQKPGKAPKLLIYWASTRESGVPSRFSGSGSGTDFTLTISSLQPEDFATYYCHQYLSSYTFGQGTKLEIK

SEQ ID NO: 9 - protein, 446 aa, synthetic construct
  source 1..446: note = Heavy chain for anti-TIM-3 antibody
QVQLVQSGAEVKKPGASVKVSCKASGYSFTGYTINWVRQAPGQGLEWMGLFNPYNGGTTYAQKFQGRVTMTVDKSTSTVYMELSSLRSEDTAVYYCARRYYGYDAMDYWGQGTLVTVSSASTKGPSVFPLAPCSRSTSESTAALGCLVKDYFPEPVTVSWNSGALTSGVHTFPAVLQSSGLYSLSSVVTVPSSSLGTKTYTCNVDHKPSNTKVDKRVESKYGPPCPPCPAPEFLGGPSVFLFPPKPKDTLMISRTPEVTCVVVDVSQEDPEVQFNWYVDGVEVHNAKTKPREEQFNSTYRVVSVLTVLHQDWLNGKEYKCKVSNKGLPSSIEKTISKAKGQPREPQVYTLPPSQEEMTKNQVSLTCLVKGFYPSDIAVEWESNGQPENNYKTTPPVLDSDGSFFLYSRLTVDKSRWQEGNVFSCSVMHEALHNHYTQKSLSLSLGK

SEQ ID NO: 10 - protein, 219 aa, synthetic construct
  source 1..219: note = Light chain for anti-TIM-3 antibody
DIQMTQSPSSLSASVGDRVTITCKSSQSVLYSSNQKNHLAWYQQKPGKAPKLLIYWASTRESGVPSRFSGSGSGTDFTLTISSLQPEDFATYYCHQYLSSYTFGQGTKLEIKRTVAAPSVFIFPPSDEQLKSGTASVVCLLNNFYPREAKVQWKVDNALQSGNSQESVTEQDSKDSTYSLSSTLTLSKADYEKHKVYACEVTHQGLSSPVTKSFNRGEC

SEQ ID NO: 11 - protein, 10 aa, synthetic construct
  source 1..10: note = VH-CDR1 for another anti-TIM-3 antibody
GFNIKDYYMH

SEQ ID NO: 12 - protein, 11 aa, synthetic construct
  source 1..11: note = VH-CDR2 for another anti-TIM-3 antibody
WIDPENDNTIY

SEQ ID NO: 13 - protein, 12 aa, synthetic construct
  source 1..12: note = VH-CDR3 for another anti-TIM-3 antibody
ARDFGYVAWLVY

SEQ ID NO: 14 - protein, 11 aa, synthetic construct
  source 1..11: note = VL-CDR1 for another anti-TIM-3 antibody
KASQNVDTAVA

SEQ ID NO: 15 - protein, 7 aa, synthetic construct
  source 1..7: note = VL-CDR2 for another anti-TIM-3 antibody
SASNRYT

SEQ ID NO: 16 - protein, 8 aa, synthetic construct
  source 1..8: note = VL-CDR3 for another anti-TIM-3 antibody
QQYSSYPT

SEQ ID NO: 17 - protein, 119 aa, synthetic construct
  source 1..119: note = VH for another anti-TIM-3 antibody
EVQLQQSGAEVVRPGALVKLSCKASGFNIKDYYMHWVRQRPEQGLEWIGWIDPENDNTIYDPKFQDRASITADTSSNTAYLQLSSLTSEDTAVYYCARDFGYVAWLVYWGQGTLVTVSA

SEQ ID NO: 18 - protein, 106 aa, synthetic construct
  source 1..106: note = VL for another anti-TIM-3 antibody
DIVMTQSQEFMSTSVGDRVSITCKASQNVDTAVAWYQQKPGQSPKLLIYSASNRYTGVPDRFTGTGSGTDFTLTINNMQSEDLADYFCQQYSSYPTFGGRTKLEIK

SEQ ID NO: 19 - protein, 446 aa, synthetic construct
  source 1..446: note = Heavy chain for another anti-TIM-3 antibody
EVQLQQSGAEVVRPGALVKLSCKASGFNIKDYYMHWVRQRPEQGLEWIGWIDPENDNTIYDPKFQDRASITADTSSNTAYLQLSSLTSEDTAVYYCARDFGYVAWLVYWGQGTLVTVSAASTKGPSVFPLAPCSRSTSESTAALGCLVKDYFPEPVTVSWNSGALTSGVHTFPAVLQSSGLYSLSSVVTVPSSSLGTKTYTCNVDHKPSNTKVDKRVESKYGPPCPPCPAPEFLGGPSVFLFPPKPKDTLMISRTPEVTCVVVDVSQEDPEVQFNWYVDGVEVHNAKTKPREEQFNSTYRVVSVLTVLHQDWLNGKEYKCKVSNKGLPSSIEKTISKAKGQPREPQVYTLPPSQEEMTKNQVSLTCLVKGFYPSDIAVEWESNGQPENNYKTTPPVLDSDGSFFLYSRLTVDKSRWQEGNVFSCSVMHEALHNHYTQKSLSLSLGK

SEQ ID NO: 20 - protein, 213 aa, synthetic construct
  source 1..213: note = Light chain for another anti-TIM-3 antibody
DIVMTQSQEFMSTSVGDRVSITCKASQNVDTAVAWYQQKPGQSPKLLIYSASNRYTGVPDRFTGTGSGTDFTLTINNMQSEDLADYFCQQYSSYPTFGGRTKLEIKRTVAAPSVFIFPPSDEQLKSGTASVVCLLNNFYPREAKVQWKVDNALQSGNSQESVTEQDSKDSTYSLSSTLTLSKADYEKHKVYACEVTHQGLSSPVTKSFNRGEC

SEQ ID NO: 21 - protein, 12 aa, synthetic construct
  source 1..12: note = VH-CDR3 for anti-TIM-3 antibody
ARRYYGYDAMDY

SEQ ID NO: 22 - protein, 440 aa, synthetic construct
  source 1..440: note = Heavy chain of TSR022
EVQLLESGGGLVQPGGSLRLSCAAASGFTFSSYDMSWVRQAPGKGLDWVSTISGGGTYTYYQDSVKGRFTISRDNSKNTLYLQMNSLRAEDTAVYYCASMDYWGQGTTVTVSSASTKGPSVFPLAPCSRSTSESTAALGCLVKDYFPEPVTVSWNSGALTSGVHTFPAVLQSSGLYSLSSVVTVPSSSLGTKTYTCNVDHKPSNTKVDKRVESKYGPPCPPCPAPEFLGGPSVFLFPPKPKDTLMISRTPEVTCVVVDVSQEDPEVQFNWYVDGVEVHNAKTKPREEQFNSTYRVVSVLTVLHQDWLNGKEYKCKVSNKGLPSSIEKTISKAKGQPREPQVYTLPPSQEEMTKNQVSLTCLVKGFYPSDIAVEWESNGQPENNYKTTPPVLDSDGSFFLYSRLTVDKSRWQEGNVFSCSVMHEALHNHYTQKSLSLSLGK

SEQ ID NO: 23 - protein, 214 aa, synthetic construct
  source 1..214: note = Light chain of TSR022
DIQMTQSPSSLSASVGDRVTITCRASQSIRRYLNWYHQKPGKAPKLLIYGASTLQSGVPSRFSGSGSGTDFTLTISSLQPEDFAVYYCQQSHSAPLTFGGGTKVEIKRTVAAPSVFIFPPSDEQLKSGTASVVCLLNNFYPREAKVQWKVDNALQSGNSQESVTEQDSKDSTYSLSSTLTLSKADYEKHKVYACEVTHQGLSSPVTKSFNRGEC